European Patent Specification EP 3 284 830 B1, published April 1, 2026. Title: A biomarker for mental disease. Applicant: National Center of Neurology and Psychiatry;Kabushiki Kaisha Yakult Honsha. Application JP2015-083936. The sequence listing filed with the application follows.

SEQUENCE LISTING (36 sequences)

SEQ ID NO: 1 - DNA, 17 bp, Artificial Sequence
  Designed primer based on Atopobium cluster
gggttgagagaccgacc

SEQ ID NO: 2 - DNA, 18 bp, Artificial Sequence
  Designed primer based on Atopobium cluster
cggrgcttcttctgcagg

SEQ ID NO: 3 - DNA, 17 bp, Artificial Sequence
  Designed primer based on Lactobacillus
accgcatggttcttggc

SEQ ID NO: 4 - DNA, 20 bp, Artificial Sequence
  Designed primer based on Lactobacillus
ccgacaacagttactctgcc

SEQ ID NO: 5 - DNA, 27 bp, Artificial Sequence
  Designed primer based on Lactobacillus
gatgcatagccgagttgagagactgat

SEQ ID NO: 6 - DNA, 25 bp, Artificial Sequence
  Designed primer based on Lactobacillus
taaaggccagttactacctctatcc

SEQ ID NO: 7 - DNA, 17 bp, Artificial Sequence
  Designed primer based on Lactobacillus
accgcatggttcttggc

SEQ ID NO: 8 - DNA, 20 bp, Artificial Sequence
  Designed primer based on Lactobacillus
ccgacaacagttactctgcc

SEQ ID NO: 9 - DNA, 27 bp, Artificial Sequence
  Designed primer based on Lactobacillus
gatgcatagccgagttgagagactgat

SEQ ID NO: 10 - DNA, 25 bp, Artificial Sequence
  Designed primer based on Lactobacillus
taaaggccagttactacctctatcc

SEQ ID NO: 11 - DNA, 25 bp, Artificial Sequence
  Designed primer based on Lactobacillus
ctctggtattgattggtgcttgcat

SEQ ID NO: 12 - DNA, 24 bp, Artificial Sequence
  Designed primer based on Lactobacillus
gttcgccactcactcaaatgtaaa

SEQ ID NO: 13 - DNA, 16 bp, Artificial Sequence
  Designed primer based on Lactobacillus
gaacgcaytggcccaa

SEQ ID NO: 14 - DNA, 19 bp, Artificial Sequence
  Designed primer based on Lactobacillus
tccattgtggccgatcagt

SEQ ID NO: 15 - DNA, 21 bp, Artificial Sequence
  Designed primer based on Lactobacillus
caccgaatgcttgcaytcacc

SEQ ID NO: 16 - DNA, 19 bp, Artificial Sequence
  Designed primer based on Lactobacillus
gccgcgggtccatccaaaa

SEQ ID NO: 17 - DNA, 22 bp, Artificial Sequence
  Designed primer based on Lactobacillus
cataaaacctamcaccgcatgg

SEQ ID NO: 18 - DNA, 27 bp, Artificial Sequence
  Designed primer based on Lactobacillus
tcagttactatcagatacrttcttctc

SEQ ID NO: 19 - DNA, 24 bp, Artificial Sequence
  Designed primer based on Lactobacillus
attttgtttgaaaggtggcttcgg

SEQ ID NO: 20 - DNA, 25 bp, Artificial Sequence
  Designed primer based on Lactobacillus
acccttgaacagttactctcaaagg

SEQ ID NO: 21 - DNA, 17 bp, Artificial Sequence
  Designed primer based on Bifidobacterium
ctcctggaaacgggtgg

SEQ ID NO: 22 - DNA, 22 bp, Artificial Sequence
  Designed primer based on Bifidobacterium
ggtgttcttcccgatatctaca

SEQ ID NO: 23 - DNA, 21 bp, Artificial Sequence
  Designed primer based on Bacteroides fragilis group
ayagcctttcgaaagraagat

SEQ ID NO: 24 - DNA, 21 bp, Artificial Sequence
  Designed primer based on Bacteroides fragilis group
ccagtatcaactgcaatttta

SEQ ID NO: 25 - DNA, 20 bp, Artificial Sequence
  Designed primer based on Enterococcus
atcagagggggataacactt

SEQ ID NO: 26 - DNA, 21 bp, Artificial Sequence
  Designed primer based on Enterococcus
actctcatccttgttcttctc

SEQ ID NO: 27 - DNA, 20 bp, Artificial Sequence
  Designed primer based on Clostridium coccoides group
aaatgacggtacctgactaa

SEQ ID NO: 28 - DNA, 22 bp, Artificial Sequence
  Designed primer based on Clostridium coccoides group
ctttgagtttcattcttgcgaa

SEQ ID NO: 29 - DNA, 16 bp, Artificial Sequence
  Designed primer based on Clostridium leptum subgroup
gcacaagcagtggagt

SEQ ID NO: 30 - DNA, 18 bp, Artificial Sequence
  Designed primer based on Clostridium leptum subgroup
cttcctccgttttgtcaa

SEQ ID NO: 31 - DNA, 30 bp, Artificial Sequence
  Designed primer based on Staphylococcus
tttgggctacacacgtgctacaatggacaa

SEQ ID NO: 32 - DNA, 24 bp, Artificial Sequence
  Designed primer based on Staphylococcus
aacaactttatgggatttgcwtga

SEQ ID NO: 33 - DNA, 18 bp, Artificial Sequence
  Designed primer based on Clostridium perfringens
gggggtttcaacacctcc

SEQ ID NO: 34 - DNA, 18 bp, Artificial Sequence
  Designed primer based on Clostridium perfringens
gcaagggatgtcaagtgt

SEQ ID NO: 35 - DNA, 23 bp, Artificial Sequence
  Designed primer based on Enterobacteriaceae
tgccgtaacttcgggagaaggca

SEQ ID NO: 36 - DNA, 22 bp, Artificial Sequence
  Designed primer based on Enterobacteriaceae
tcaaggaccagtgttcagtgtc